European Patent Specification EP 3 901 246 B1, published July 17, 2024. Title: Filmentous Fungal Biomats, Methods of their Production and Methods of their Use. Applicant: The Fynder Group, Inc. The sequence listing filed with the application follows.

SEQUENCE LISTING (3 sequences)

SEQ ID NO: 1 - DNA, 1077 bp, Strain MK7
atgatcactggtacttcccaggccgattgcgccattctcatcattgccgccggtactggtgagttcgaggctggtatctccaaggatggccagacccgtgagcacgctcttcttgcctacacccttggtgtcaagaacctcatcgtcgccatcaacaagatggacaccaccaagtggtctgaggcccgttaccaggagatcatcaaggagacctcctccttcatcaagaaggtcggctacaaccccaaggctgtcgctttcgtccccatctccggtttcaacggtgacaacatgcttaccccctccaccaactgcccctggtacaagggttgggagcgtgagatcaagtccggcaagctcaccggcaagaccctcctcgaggccattgactccatcgagcctcccaagcgtcccgttgacaagcccctccgtcttcccctccaggatgtctacaagatcggtggtattggaacggttcccgtcggccgtattgagactggtgtcatcaagcccggtatggtcgttaccttcgctccctccaacgtcaccactgaagtcaagtccgtcgagatgcaccacgagcagctcagtgagggccagcccggtgacaacgttggtttcaacgtgaagaacgtctccgtcaaggacatccgacgtggtaacgtcgctggtgactccaagaacgaccccccccagggtgccgcttctttcaccgcccaggtcatcgtcctcaaccaccccggccaggtcggtgctggttacgctcccgtcctcgattgccacactgcccacattgcctgcaagttcgccgagatccaggagaagatcgaccgccgaaccggtaaggctactgaggccgctcccaagttcatcaagtctggtgactccgccatcgtcaagatggttccctccaagcccatgtgtgtcgaggctttcactgactaccctcctctgggtcgtttcgccgtccgtgacatgcgacagactgtcgccgtcggtgtcatcaaggccgtcgagaagtccaccggtgctgctggcaaggtcaccaagtccgctgccaaggccgccaagaaataa

SEQ ID NO: 2 - DNA, 480 bp, Strain MK7
gtggatcttgagcccggtcctcaggatgccatccgcgccgggcccctaggccagcttttccgccccgacaacttcgtcgccggaaatgccagcgccggtaacaactgggccaagggtcattacaccgaaggtgctgagctcgttgaggaggccatcgatgttgtgcgacacgaggttgagaactgtgaccatcttcagggtttccagctcacccactctctcggcggtggtaccggttctggtatgggaacgcttcttctgtcgaaaatccgtgaggagtttcccgatcgcatgatggctactttttccgttatgccttcgcctaaggtttctgataccgttgtcgaaccttacaacgccactttgtcattgaaccagcttgtcgagaactccgatgagaccttctgtatcgataacgaggctttgtacgacatttacgagaagaccctgaagattgctgatccttcttacgccgatctc

SEQ ID NO: 3 - DNA, 962 bp, Strain MK7
ccgcggggaatactacctgatccgaggtcacattcagagttgggggtttacggcttggccgcgccgcgtaccagttgcgagggttttactactacgcaatggaagctgcagcgagaccgccactagatttcggggccggcttgccgcaagggctcgccgatccccaacaccaaacccgggggcttgagggttgaaatgacgctcgaacaggcatgcccgccagaatactggcgggcgcaatgtgcgttcaaagattcgatgattcactgaattctgcaattcacattacttatcgcattttgctgcgttcttcatcgatgccagaaccaagagatccgttgttgaaagttttgatttatttatggttttactcagaagttacatatagaaacagagtttaggggtcctctggcgggccgtcccgttttaccgggagcgggctgatccgccgaggcaacaattggtatgttcacaggggtttgggagttgtaaactcggtaatgatccctccgcagttctcacctacggataggatcattaccgagtttacaactcccaaacccctgtgaacatacccattgttgcctcggccggatcagcccgctcccggttaaaacgggacggcccgccagagtacccctaaactctgtttctatatgtaacttctgagtaaaaccataaataaatcaaaactttcaacacgcatctcttgcttctgtcatcgatgaagaacgcagcaaaatgcgatagtcatgtgattgcacattcagtgaatcatcgatcttgacgcacattgcgcctgcagtattctggcggtcatgcctgttcgagcgtcattcagccctcagccctcggttgtgttcgggatcggcgagtcctgcgccagcgaccggatcagtggcgtctgcctgcgcctccattgcggttagagttaagccctcgcccacttgttttacgctaac